European Patent Application EP 4 610 236 A1, published September 3, 2025. Title: Yeasts for the treatment of saline wastewater comprising formate. Applicant: Covestro Deutschland AG. Application EP. The sequence listing filed with the application follows.

SEQUENCE LISTING (4 sequences)

SEQ ID NO: 1 - protein, 364 aa, Candida boidinii
MKIVLVLYDAGKHAADEEKLYGCTENKLGIANWLKDQGHELITTSDKEGETSELDKHIPDADIIITTPFHPAYITKERLDKAKNLKLVVVAGVGSDHIDLDYINQTGKKISVLEVTGSNVVSVAEHVVMTMLVLVRNFVPAHEQIINHDWEVAAIAKDAYDIEGKTIATIGAGRIGYRVLERLLPFNPKELLYYDYQALPKEAEEKVGARRVENIEELVAQADIVTVNAPLHAGTKGLINKELLSKFKKGAWLVNTARGAICVAEDVAAALESGQLRGYGGDVWFPQPAPKDHPWRDMRNKYGAGNAMTPHYSGTTLDAQTRYAEGTKNILESFFTGKFDYRPQDIILLNGEYVTKAYGKHDKK

SEQ ID NO: 2 - protein, 362 aa, Hansenula polymorpha
MKVVLVLYDAGKHAQDEERLYGCTENALGIRDWLEKQGHELVVTSDKEGQNSVLEKNISDADVIISTPFHPAYITKERIDKAKKLKLLVVAGVGSDHIDLDYINQSGRDISVLEVTGSNVVSVAEHVVMTMLVLVRNFVPAHEQIISGGWNVAEIAKDSFDIEGKVIATIGAGRIGYRVLERLVAFNPKELLYYDYQSLSKEAEEKVGARRVHDIKELVAQADIVTINCPLHAGSKGLVNAELLKHFKKGAWLVNTARGAICVAEDVAAAVKSGQLRGYGGDVWFPQPAPKDHPWRSMANKYGAGNAMTPHYSGSVIDAQVRYAQGTKNILESFFTQKFDYRPQDIILLNGKYKTKSYGADK

SEQ ID NO: 3 - protein, 576 aa, Schwanniomyces vanrijiae
MVQSHYDFVIVGGGTAGNTVAGRLAENPNVTVLVVEAGVANSADLPEITTPSNAMNLRGSKHDWAYKTTLVKRDDYERIEKPNTRGKALGGSSSLNYFTWIPGCKPTFDRWAEYGGEEWTWDPLVPYLRKSATYHDDTGLYNPELKKLGAGGPIPISHSELVEELEPFRENLIKAWKSTGKPFTENIYDGEMIGLNHCISTIYHGKRSGSFLFVKNRPNITIIPEVHSKNLIIDASNTAKGVVVIDKEGNEHSFYATREVILSQGVFESPKLLMLSGVGPRKELESNGIEVKVESRHVGQNLLDHPGVPFVLQVKDDICVDDILMRQNEKNKAAHVQYQKDGSGPVGSGLLELVGFPRIDEYFEKDPLYRERKAANGGKDPFCPEGQPHFELDFVGMYGTAFQWHFPTPKKGSHITIVVDLVRPVSEGGEVTLNSADPLEQPKINLNFFADELDIVGMREGIRFTYDLLTKGDGFKDLVVKEFPWEMPLDDDKEMRRAVLDRCQTAFHPCGTNRLSKNIEQGVVDPALKVHGVKNLRVIDASIIPVIPDCRIQNSVYMIGEKGADLIKAAHKDLYN

SEQ ID NO: 4 - protein, 578 aa, Aspergillus oryzae
MATDGSHFDFVIVGGGTAGNTVAGRLAENPNVTVLIVEAGIGNPEDIPEITTPSSAMDLRNSKYDWAYKTTMVRRDDYERIEKPNTRGKTLGGSSSLNYFTWVPGHKATFDQWEEFGGKEWTWDPLVPYLRKSATYHDDPRLYSPELEKIGGGGPIPISHAELIDEMAPFRENLTKAWKSMGQPLIENIYDGEMDGLTHCCDTIYRGQRSGSFLFVKNKPNITIVPEVHSKRLIINEADRTCKGVTVVTAAGNELNFFADREVILSQGVFETPKLLMLSGIGPTRELSRHGINTIVDSRHVGQNLMDHPGVPFVLRVKDGFGMDDVLLRHGPKRDAVVSAYNKNRSGPVGSGLLELVGFPRIDKYLEKDAEYRKAKAANGGKDPFSPLGQPHFELDFVCMFGTAFQWHFPTPKTGDHLTVVVDLVRPISDPGEVTLNSADPFQQPNINLNFFANDLDIIAMREGIRFSYDLLFKGEGFKDLVESEYPWEMPLDSDKEMHRAVLDRCQTAFHPTGTARLSKNIDQGVVDPKLKVHGIKKLRVADASVIPIIPDCRIQNSVYAVGEKCADMIKAEHKDLY